European Patent Specification EP 4 053 160 B1, published September 10, 2025. Title: HUMAN COLLAGEN 17-TYPE POLYPEPTIDE, PRODUCTION METHOD THEREFOR AND USE THEREOF. Applicant: SHANXI JINBO BIO-PHARMACEUTICAL CO., LTD. The sequence listing filed with the application follows.

SEQUENCE LISTING (9 sequences)

SEQ ID NO: 1 - protein, 69 aa, Artificial Sequence
  C17A
GSPGPKGDMGSPGPKGDRGFPGTPGIPGPLGHPGPQGPKGQKGSVGDPGMEGPMGQRGREGPMGPRGEA

SEQ ID NO: 2 - protein, 63 aa, Artificial Sequence
  C17B
GLQGLRGEVGLPGVKGDKGPMGPPGPKGDQGEKGPRGLTGEPGMRGLPGAVGEPGAKGAMGPA

SEQ ID NO: 3 - protein, 119 aa, Artificial Sequence
  C17C1
GADFAGDLDYNELAVRVSESMQRQGLLQGMAYTVQGPPGQPGPQGPPGISKVFSAYSNVTADLMDFFQTYGAIQGPPGQKGEMGTPGPKGDRGPAGPPGHPGPPGPRGHKGEKGDKGDQ

SEQ ID NO: 4 - protein, 207 aa, Artificial Sequence
  C17A3
GSPGPKGDMGSPGPKGDRGFPGTPGIPGPLGHPGPQGPKGQKGSVGDPGMEGPMGQRGREGPMGPRGEAGSPGPKGDMGSPGPKGDRGFPGTPGIPGPLGHPGPQGPKGQKGSVGDPGMEGPMGQRGREGPMGPRGEAGSPGPKGDMGSPGPKGDRGFPGTPGIPGPLGHPGPQGPKGQKGSVGDPGMEGPMGQRGREGPMGPRGEA

SEQ ID NO: 5 - DNA, 621 bp, Artificial Sequence
  C17A3-DNA
ggtagcccaggtccaaaaggtgatatgggaagcccaggtccgaaaggtgatcgtggttttccgggtacaccaggtattccgggtccactgggtcatccaggtccgcaaggtccgaaaggccagaaaggtagcgtgggtgatccgggtatggaagggcctatggggcagcgtgggcgtgaagggccgatgggtccgcgtggtgaagcaggtagcccggggcctaaaggggatatggggagtccgggtccgaaaggggatcgtggatttccgggtacgccgggtatcccgggtccgctgggtcatccgggtccgcaagggcctaaaggtcagaaaggtagtgtgggtgatcctggtatggaaggtccgatgggtcagcgtggtcgtgagggtccgatgggaccgcgtggtgaggctggtagccctggtccgaaaggagatatgggtagcccgggtccgaaaggtgaccgtggttttcctggtacaccgggtattccagggcctctgggtcatcctggtcctcagggtccgaaaggtcagaaagggagtgtgggagatccgggtatggagggtccgatggggcagcgcggtcgtgaaggtccgatgggcccgcgtggtgaagcc

SEQ ID NO: 6 - protein, 189 aa, Artificial Sequence
  C17B3
GLQGLRGEVGLPGVKGDKGPMGPPGPKGDQGEKGPRGLTGEPGMRGLPGAVGEPGAKGAMGPAGLQGLRGEVGLPGVKGDKGPMGPPGPKGDQGEKGPRGLTGEPGMRGLPGAVGEPGAKGAMGPAGLQGLRGEVGLPGVKGDKGPMGPPGPKGDQGEKGPRGLTGEPGMRGLPGAVGEPGAKGAMGPA

SEQ ID NO: 7 - DNA, 567 bp, Artificial Sequence
  C17B3-DNA
ggtctgcagggtctgcgtggtgaagtaggactgccgggtgtgaaaggagataaaggaccaatgggtccaccaggaccaaaaggagatcaaggagaaaaaggaccacgtggtctgacaggtgaaccgggtatgcgtgggctgccgggagcagttggagaaccgggagcaaaaggagcaatgggtccagcaggactgcagggtctgcgcggtgaagtgggactgcctggtgttaaaggggataaagggccgatgggtccgccgggtccgaaaggagatcagggagaaaaagggccgcgtggtctgaccggtgaaccgggaatgcgtggtctgccgggggctgtgggtgagccaggtgcaaaaggtgcaatgggtcctgcaggtctgcaaggactgcgtggagaagtgggtctgcctggtgtgaaaggtgataaaggtccgatgggtcctccgggtccgaaaggtgatcagggtgaaaaaggtccgcgtggtctgacgggtgaaccgggcatgcgtggtctgcctggggcagttggtgaaccgggggcaaaaggtgctatggggccggca

SEQ ID NO: 8 - DNA, 357 bp, Artificial Sequence
  C17C1-DNA
ggtgcagattttgcaggtgatctggattataatgaactggcagttcgtgttagcgaaagcatgcagcgtcagggactgctgcagggaatggcatataccgttcagggtccgccgggtcagccgggtcctcaaggtcctcctggtattagcaaagtttttagtgcatattcaaacgtgacggcagatctgatggatttttttcagacgtatggtgcaattcagggtcctcctgggcaaaaaggtgaaatgggtacacctggtccgaaaggcgatcgtggtccggccggtccgccgggccaccctggtcctcctggccctcgtggtcataaaggtgagaaaggtgataaaggtgatcaa

SEQ ID NO: 9 - protein, 1497 aa, Artificial Sequence
  COL17A1
MDVTKKNKRDGTEVTERIVTETVTTRLTSLPPKGGTSNGYAKTASLGGGSRLEKQSLTHGSSGYINSTGSTRGHASTSSYRRAHSPASTLPNSPGSTFERKTHVTRHAYEGSSSGNSSPEYPRKEFASSSTRGRSQTRESEIRVRLQSASPSTRWTELDDVKRLLKGSRSASVSPTRNSSNTLPIPKKGTVETKIVTASSQSVSGTYDATILDANLPSHVWSSTLPAGSSMGTYHNNMTTQSSSLLNTNAYSAGSVFGVPNNMASCSPTLHPGLSTSSSVFGMQNNLAPSLTTLSHGTTTTSTAYGVKKNMPQSPAAVNTGVSTSAACTTSVQSDDLLHKDCKFLILEKDNTPAKKEMELLIMTKDSGKVFTASPASIAATSFSEDTLKKEKQAAYNADSGLKAEANGDLKTVSTKGKTTTADIHSYGSSGGGGSGGGGGVGGAGGGPWGPAPAWCPCGSCCSWWKWLLGLLLTWLLLLGLLFGLIALAEEVRKLKARVDELERIRRSILPYGDSMDRIEKDRLQGMAPAAGADLDKIGLHSDSQEELWMFVRKKLMMEQENGNLRGSPGPKGDMGSPGPKGDRGFPGTPGIPGPLGHPGPQGPKGQKGSVGDPGMEGPMGQRGREGPMGPRGEAGPPGSGEKGERGAAGEPGPHGPPGVPGSVGPKGSSGSPGPQGPPGPVGLQGLRGEVGLPGVKGDKGPMGPPGPKGDQGEKGPRGLTGEPGMRGLPGAVGEPGAKGAMGPAGPDGHQGPRGEQGLTGMPGIRGPPGPSGDPGKPGLTGPQGPQGLPGTPGRPGIKGEPGAPGKIVTSEGSSMLTVPGPPGPPGAMGPPGPPGAPGPAGPAGLPGHQEVLNLQGPPGPPGPRGPPGPSIPGPPGPRGPPGEGLPGPPGPPGSFLSNSETFLSGPPGPPGPPGPKGDQGPPGPRGHQGEQGLPGFSTSGSSSFGLNLQGPPGPPGPQGPKGDKGDPGVPGALGIPSGPSEGGSSSTMYVSGPPGPPGPPGPPGSISSSGQEIQQYISEYMQSDSIRSYLSGVQGPPGPPGPPGPVTTITGETFDYSELASHVVSYLRTSGYGVSLFSSSISSEDILAVLQRDDVRQYLRQYLMGPRGPPGPPGASGDGSLLSLDYAELSSRILSYMSSSGISIGLPGPPGPPGLPGTSYEELLSLLRGSEFRGIVGPPGPPGPPGIPGNVWSSISVEDLSSYLHTAGLSFIPGPPGPPGPPGPRGPPGVSGALATYAAENSDSFRSELISYLTSPDVRSFIVGPPGPPGPQGPPGDSRLLSTDASHSRGSSSSSHSSSVRRGSSYSSSMSTGGGGAGSLGAGGAFGEAAGDRGPYGTDIGPGGGYGAAAEGGMYAGNGGLLGADFAGDLDYNELAVRVSESMQRQGLLQGMAYTVQGPPGQPGPQGPPGISKVFSAYSNVTADLMDFFQTYGAIQGPPGQKGEMGTPGPKGDRGPAGPPGHPGPPGPRGHKGEKGDKGDQVYAGRRRRRSIAVKP